European Patent Application EP 4 450 973 A1, published October 23, 2024. Title: 老年痴呆症诊断及治疗的新靶点及其应用. Applicant: 上海佳文英莉生物技术有限公司. The sequence listing filed with the application follows.

SEQUENCE LISTING (37 sequences)

SEQ ID NO: 1 - protein, 40 aa, synthetic construct
LYLIYSQVLFKGQGCPSTHVLLTHTISRIAVSYQTKVNLL

SEQ ID NO: 2 - protein, 30 aa, synthetic construct
KGQGCPSTHVLLTHTISRIAVSYQTKVNLL

SEQ ID NO: 3 - protein, 30 aa, synthetic construct
ALLANGVELRDNQLVVPSEGLYLIYSQVLF

SEQ ID NO: 4 - protein, 31 aa, synthetic construct
SQVLFKGQGCPSTHVLLTHTISRIAVSYQTK

SEQ ID NO: 5 - protein, 30 aa, synthetic construct
TPEGAEAKPWYEPIYLGGVFQLEKGDRLSA

SEQ ID NO: 6 - protein, 10 aa, synthetic construct
KGQGCPSTHV

SEQ ID NO: 7 - protein, 10 aa, synthetic construct
GQGCPSTHVL

SEQ ID NO: 8 - protein, 10 aa, synthetic construct
QGCPSTHVLL

SEQ ID NO: 9 - protein, 10 aa, synthetic construct
GCPSTHVLLT

SEQ ID NO: 10 - protein, 10 aa, synthetic construct
CPSTHVLLTH

SEQ ID NO: 11 - protein, 10 aa, synthetic construct
PSTHVLLTHT

SEQ ID NO: 12 - protein, 10 aa, synthetic construct
STHVLLTHTI

SEQ ID NO: 13 - protein, 10 aa, synthetic construct
THVLLTHTIS

SEQ ID NO: 14 - protein, 10 aa, synthetic construct
HVLLTHTISR

SEQ ID NO: 15 - protein, 10 aa, synthetic construct
VLLTHTISRI

SEQ ID NO: 16 - protein, 10 aa, synthetic construct
LLTHTISRIA

SEQ ID NO: 17 - protein, 10 aa, synthetic construct
LTHTISRIAV

SEQ ID NO: 18 - protein, 10 aa, synthetic construct
THTISRIAVS

SEQ ID NO: 19 - protein, 10 aa, synthetic construct
HTISRIAVSY

SEQ ID NO: 20 - protein, 10 aa, synthetic construct
TISRIAVSYQ

SEQ ID NO: 21 - protein, 10 aa, synthetic construct
ISRIAVSYQT

SEQ ID NO: 22 - protein, 10 aa, synthetic construct
SRIAVSYQTK

SEQ ID NO: 23 - protein, 10 aa, synthetic construct
RIAVSYQTKV

SEQ ID NO: 24 - protein, 10 aa, synthetic construct
IAVSYQTKVN

SEQ ID NO: 25 - protein, 10 aa, synthetic construct
AVSYQTKVNL

SEQ ID NO: 26 - protein, 10 aa, synthetic construct
VSYQTKVNLL

SEQ ID NO: 27 - protein, 20 aa, synthetic construct
KGQGCPSTHVLLTHTISRIA

SEQ ID NO: 28 - protein, 20 aa, synthetic construct
GQGCPSTHVLLTHTISRIAV

SEQ ID NO: 29 - protein, 20 aa, synthetic construct
QGCPSTHVLLTHTISRIAVS

SEQ ID NO: 30 - protein, 20 aa, synthetic construct
GCPSTHVLLTHTISRIAVSY

SEQ ID NO: 31 - protein, 20 aa, synthetic construct
CPSTHVLLTHTISRIAVSYQ

SEQ ID NO: 32 - protein, 20 aa, synthetic construct
PSTHVLLTHTISRIAVSYQT

SEQ ID NO: 33 - protein, 20 aa, synthetic construct
STHVLLTHTISRIAVSYQTK

SEQ ID NO: 34 - protein, 20 aa, synthetic construct
THVLLTHTISRIAVSYQTKV

SEQ ID NO: 35 - protein, 20 aa, synthetic construct
HVLLTHTISRIAVSYQTKVN

SEQ ID NO: 36 - protein, 20 aa, synthetic construct
VLLTHTISRIAVSYQTKVNL

SEQ ID NO: 37 - protein, 20 aa, synthetic construct
LLTHTISRIAVSYQTKVNLL